European Patent Application EP 4 253 540 A1, published October 4, 2023. Title: ANTISENSE NUCLEIC ACID AND USE THEREOF. Applicant: NIIGATA UNIVERSITY. The sequence listing filed with the application follows.

SEQUENCE LISTING (33 sequences)

SEQ ID NO: 1 - DNA, 1015 bp, Homo sapiens
atatccaatgccgaacctaagcacaatagcaatagacagttagaaagaagtggaagatttggtggtaatccaggtggctttgggaatcagggtggatttggtaatagcagagggggtggagctggtttgggaaacaatcaaggtagtaatatgggtggtgggatgaactttggtgcgttcagcattaatccagccatgatggctgccgcccaggcagcactacagagcagttggggtatgatgggcatgttagccagccagcagaaccagtcaggcccatcgggtaataaccaaaaccaaggcaacatgcagagggagccaaaccaggccttcggttctggaaataactcttatagtggctctaattctggtgcagcaattggttggggatcagcatccaatgcagggtcgggcagtggttttaatggaggctttggctcaagcatggattctaagtcttctggctggggaatgtagacagtggggttgtggttggttggtatagaatggtgggaattcaaatttttctaaactcatggtaagtatattgtaaaatacatatgtactaagaattttcaaaattggtttgttcagtgtggagtatattcagcagtatttttgacatttttctttagaaaaaggaagagctaaaggaattttataagttttgttacatgaaaggttgaaatattgagtggttgaaagtgaactgctgtttgcctgattggtaaaccaacacactacaattgatatcaaaaggtttctcctgtaatattttatccctggacttgtcaagtgaattctttgcatgttcaaaacggaaaccattgattagaactacattctttaccccttgttttaatttgaaccccaccatatggatttttttccttaagaaaatctccttttaggagatcatggtgtcacagtgtttggttcttttgttttgttttttaacacttgtctcccctcatacacaaaagtacaatatgaagccttcatttaatctctgcag

SEQ ID NO: 2 - DNA, 25 bp, Artificial Sequence
  Synthetic nucleotides for AS2
tccaccccctctgctattaccaaat

SEQ ID NO: 3 - DNA, 25 bp, Artificial Sequence
  Synthetic nucleotides for AS4
tgctgaacgcaccaaagttcatccc

SEQ ID NO: 4 - DNA, 25 bp, Artificial Sequence
  Synthetic nucleotides for AS5
gctaacatgcccatcataccccaac

SEQ ID NO: 5 - DNA, 24 bp, Artificial Sequence
  Synthetic nucleotides for AS5.1
cataccccaactgctctgtagtgc

SEQ ID NO: 6 - DNA, 25 bp, Artificial Sequence
  Synthetic nucleotides for AS5.2
ggttttggttattacccgatgggcc

SEQ ID NO: 7 - DNA, 25 bp, Artificial Sequence
  Synthetic nucleotides for AS6.1
gcctccattaaaaccactgcccgac

SEQ ID NO: 8 - DNA, 20 bp, Artificial Sequence
  Synthetic nucleotides for forward primer of TDP-43 mRNA intron 6
gcgctgtacagaggacatga

SEQ ID NO: 9 - DNA, 18 bp, Artificial Sequence
  Synthetic nucleotides for reverse primer of TDP-43 mRNA intron 6
gcctgtgatgcgtgatga

SEQ ID NO: 10 - DNA, 20 bp, Artificial Sequence
  Synthetic nucleotides for reverse primer of TDP-43 mRNA intron 6
agttccatctcaaaagggtc

SEQ ID NO: 11 - DNA, 25 bp, Artificial Sequence
  Synthetic nucleotides for AS1
aagccacctggattaccaccaaatc

SEQ ID NO: 12 - DNA, 25 bp, Artificial Sequence
  Synthetic nucleotides for AS2.1
cctctgctattaccaaatccaccct

SEQ ID NO: 13 - DNA, 25 bp, Artificial Sequence
  Synthetic nucleotides for AS3
tgattgtttcccaaaccagctccac

SEQ ID NO: 14 - DNA, 25 bp, Artificial Sequence
  Synthetic nucleotides for AS6
aattgctgcaccagaattagagcca

SEQ ID NO: 15 - DNA, 25 bp, Artificial Sequence
  Synthetic nucleotides for AS7
actccatgaaataaagagtagcgga

SEQ ID NO: 16 - DNA, 20 bp, Artificial Sequence
  Synthetic nucleotides for forward primer of TDP-43 mRNA intron 6
cagagcttttgccttcgtca

SEQ ID NO: 17 - DNA, 18 bp, Artificial Sequence
  Synthetic nucleotides for reverse primer of TDP-43 mRNA intron 6
caaagacgcagcctgtgc

SEQ ID NO: 18 - DNA, 22 bp, Artificial Sequence
  Synthetic nucleotides for forward primer of TDP-43 mRNA exon3-4
aactgagcaggatctgaaagac

SEQ ID NO: 19 - DNA, 21 bp, Artificial Sequence
  Synthetic nucleotides for reverse primer of TDP-43 mRNA exon3-4
cgaacaaagccaaaccctttc

SEQ ID NO: 20 - DNA, 9 bp, Artificial Sequence
  Synthetic nucleotides for a part of probe (5' region) of TDP-43 mRNA exon 3-4
tggagaggt

SEQ ID NO: 21 - DNA, 17 bp, Artificial Sequence
  Synthetic nucleotides for a part of probe (3' region) of TDP-43 mRNA exon 3-4
tcttatggttcaggtca

SEQ ID NO: 22 - DNA, 19 bp, Artificial Sequence
  Synthetic nucleotides for forward primer of TDP-43 mRNA intron 6
aggtggctttgggaatcag

SEQ ID NO: 23 - DNA, 20 bp, Artificial Sequence
  Synthetic nucleotides for reverse primer of TDP-43 mRNA intron 6
caccaaagttcatccctcca

SEQ ID NO: 24 - DNA, 9 bp, Artificial Sequence
  Synthetic nucleotides for a part of probe (5' region) of TDP-43 mRNA intron 6
tggagctgg

SEQ ID NO: 25 - DNA, 15 bp, Artificial Sequence
  Synthetic nucleotides for a part of probe (3' region) of TDP-43 mRNA intron 6
cttgggaaataacca

SEQ ID NO: 26 - DNA, 21 bp, Artificial Sequence
  Synthetic nucleotides for forward primer of TDP-43 mRNA intron 7
tgctgtatggtgtgtgttctc

SEQ ID NO: 27 - DNA, 20 bp, Artificial Sequence
  Synthetic nucleotides for reverse primer of TDP-43 mRNA intron 7
ccacaagctcagtccatgtt

SEQ ID NO: 28 - DNA, 9 bp, Artificial Sequence
  Synthetic nucleotides for a part of probe (5' region) of TDP-43 mRNA intron 7
agtgtggga

SEQ ID NO: 29 - DNA, 15 bp, Artificial Sequence
  Synthetic nucleotides for a part of probe (3' region) of TDP-43 mRNA intron 7
acgtgaactgaagct

SEQ ID NO: 30 - DNA, 20 bp, Artificial Sequence
  Synthetic nucleotides for forward primer of GAPDH
tgtgtccgtcgtggatctga

SEQ ID NO: 31 - DNA, 21 bp, Artificial Sequence
  Synthetic nucleotides for reverse primer of GAPDH
ttgctgttgaagtcgcaggag

SEQ ID NO: 32 - DNA, 20 bp, Artificial Sequence
  Synthetic nucleotides for forward primer of Aif1
acgaaccctctgatgtggtc

SEQ ID NO: 33 - DNA, 19 bp, Artificial Sequence
  Synthetic nucleotides for reverse primer of Aif1
cgggatggaagagagagga